European Patent Specification EP 3 524 273 B1, published June 18, 2025. Title: CYSTEINE MODIFIED ANTIBODY-DRUG CONJUGATE AND PREPARATION METHOD THEREOF. Applicant: Baili-Bio (Chengdu) Pharmaceutical Co., Ltd. The sequence listing filed with the application follows.

SEQUENCE LISTING (12 sequences)

SEQ ID NO: 1 - DNA, 990 bp, Fc DNA
gctagcaccaagggcccatcggtcttccccctggcaccctcctccaagagcacctctgggggcacagcggccctgggctgcctggtcaaggactacttccccgaaccggtgacggtgtcgtggaactcaggcgccctgaccagcggcgtgcacaccttcccggctgtcctacagtcctcaggactctactccctcagcagcgtggtgaccgtgccctccagcagcttgggcacccagacctacatctgcaacgtgaatcacaagcccagcaacaccaaggtggacaagagagttgagcccaaatcttgtgacaaaactcacacatgcccaccgtgcccagcacctgaactcctggggggaccgtcagtcttcctcttccccccaaaacccaaggacaccctcatgatctcccggacccctgaggtcacatgcgtggtggtggacgtgagccacgaagaccctgaggtcaagttcaactggtacgtggacggcgtggaggtgcataatgccaagacaaagccgcgggaggagcagtacaacagcacgtaccgtgtggtcagcgtcctcaccgtcctgcaccaggactggctgaatggcaaggagtacaagtgcaaggtctccaacaaagccctcccagcccccatcgagaaaaccatctccaaagccaaagggcagccccgagaaccacaggtgtacaccctgcccccatcccgggatgagctgaccaagaaccaggtcagcctgacctgcctggtcaaaggcttctatcccagcgacatcgccgtggagtgggagagcaatgggcagccggagaacaactacaagaccacgcctcccgtgctggactccgacggctccttcttcctctatagcaagctcaccgtggacaagagcaggtggcagcaggggaacgtcttctcatgctccgtgatgcatgaggctctgcacaaccactacacgcagaagagcctctccctgtctccgggtaaa

SEQ ID NO: 2 - protein, 330 aa, Fc
ASTKGPSVFPLAPSSKSTSGGTAALGCLVKDYFPEPVTVSWNSGALTSGVHTFPAVLQSSGLYSLSSVVTVPSSSLGTQTYICNVNHKPSNTKVDKRVEPKSCDKTHTCPPCPAPELLGGPSVFLFPPKPKDTLMISRTPEVTCVVVDVSHEDPEVKFNWYVDGVEVHNAKTKPREEQYNSTYRVVSVLTVLHQDWLNGKEYKCKVSNKALPAPIEKTISKAKGQPREPQVYTLPPSRDELTKNQVSLTCLVKGFYPSDIAVEWESNGQPENNYKTTPPVLDSDGSFFLYSKLTVDKSRWQQGNVFSCSVMHEALHNHYTQKSLSLSPGK

SEQ ID NO: 3 - DNA, 321 bp, Kappa DNA
acggtggctgcaccatctgtcttcatcttcccgccatctgatgagcagttgaaatctggaactgcctctgttgtgtgcctgctgaataacttctatcccagagaggccaaagtacagtggaaggtggataacgccctccaatcgggtaactcccaggagagtgtcacagagcaggacagcaaggacagcacctacagcctcagcagcaccctgacgctgagcaaagcagactacgagaaacacaaagtctacgcctgcgaagtcacccatcagggcctgagctcgcccgtcacaaagagcttcaacaggggagagtgttag

SEQ ID NO: 4 - protein, 106 aa, Kappa
TVAAPSVFIFPPSDEQLKSGTASVVCLLNNFYPREAKVQWKVDNALQSGNSQESVTEQDSKDSTYSLSSTLTLSKADYEKHKVYACEVTHQGLSSPVTKSFNRGEC

SEQ ID NO: 5 - DNA, 324 bp, 2A1-LC-Cys205ins Kappa DNA
acggtggctgcaccatctgtcttcatcttcccgccatctgatgagcagttgaaatctggaactgcctctgttgtgtgcctgctgaataacttctatcccagagaggccaaagtacagtggaaggtggataacgccctccaatcgggtaactcccaggagagtgtcacagagcaggacagcaaggacagcacctacagcctcagcagcaccctgacgctgagcaaagcagactacgagaaacacaaagtctacgcctgcgaagtcacccatcagggcctgagctcgccctgcgtcacaaagagcttcaacaggggagagtgttag

SEQ ID NO: 6 - protein, 107 aa, LC-Cys205ins Kappa
TVAAPSVFIFPPSDEQLKSGTASVVCLLNNFYPREAKVQWKVDNALQSGNSQESVTEQDSKDSTYSLSSTLTLSKADYEKHKVYACEVTHQGLSSPCVTKSFNRGEC

SEQ ID NO: 7 - DNA, 324 bp, LC-Cys206ins Kappa DNA
acggtggctgcaccatctgtcttcatcttcccgccatctgatgagcagttgaaatctggaactgcctctgttgtgtgcctgctgaataacttctatcccagagaggccaaagtacagtggaaggtggataacgccctccaatcgggtaactcccaggagagtgtcacagagcaggacagcaaggacagcacctacagcctcagcagcaccctgacgctgagcaaagcagactacgagaaacacaaagtctacgcctgcgaagtcacccatcagggcctgagctcgcccgtctgcacaaagagcttcaacaggggagagtgttag

SEQ ID NO: 8 - protein, 107 aa, LC-Cys206ins Kappa
TVAAPSVFIFPPSDEQLKSGTASVVCLLNNFYPREAKVQWKVDNALQSGNSQESVTEQDSKDSTYSLSSTLTLSKADYEKHKVYACEVTHQGLSSPVCTKSFNRGEC

SEQ ID NO: 9 - DNA, 993 bp, IgG1-Fc-Cys474ins Fc DNA
gctagcaccaagggcccatcggtcttccccctggcaccctcctccaagagcacctctgggggcacagcggccctgggctgcctggtcaaggactacttccccgaaccggtgacggtgtcgtggaactcaggcgccctgaccagcggcgtgcacaccttcccggctgtcctacagtcctcaggactctactccctcagcagcgtggtgaccgtgccctccagcagcttgggcacccagacctacatctgcaacgtgaatcacaagcccagcaacaccaaggtggacaagagagttgagcccaaatcttgtgacaaaactcacacatgcccaccgtgcccagcacctgaactcctggggggaccgtcagtcttcctcttccccccaaaacccaaggacaccctcatgatctcccggacccctgaggtcacatgcgtggtggtggacgtgagccacgaagaccctgaggtcaagttcaactggtacgtggacggcgtggaggtgcataatgccaagacaaagccgcgggaggagcagtacaacagcacgtaccgtgtggtcagcgtcctcaccgtcctgcaccaggactggctgaatggcaaggagtacaagtgcaaggtctccaacaaagccctcccagcccccatcgagaaaaccatctccaaagccaaagggcagccccgagaaccacaggtgtacaccctgcccccatcccgggatgagctgaccaagaaccaggtcagcctgacctgcctggtcaaaggcttctatcccagcgacatcgccgtggagtgggagagcaatgggcagccggagaacaactacaagaccacgcctcccgtgctggactccgacggctccttcttcctctatagcaagctcaccgtggacaagagcaggtggcagcaggggaacgtcttctcatgctccgtgatgcatgaggctctgcacaaccactacacgcagaagagcctctcctgcctgtctccgggtaaa

SEQ ID NO: 10 - protein, 331 aa, IgG1-Fc-Cys474ins Fc
ASTKGPSVFPLAPSSKSTSGGTAALGCLVKDYFPEPVTVSWNSGALTSGVHTFPAVLQSSGLYSLSSVVTVPSSSLGTQTYICNVNHKPSNTKVDKRVEPKSCDKTHTCPPCPAPELLGGPSVFLFPPKPKDTLMISRTPEVTCVVVDVSHEDPEVKFNWYVDGVEVHNAKTKPREEQYNSTYRVVSVLTVLHQDWLNGKEYKCKVSNKALPAPIEKTISKAKGQPREPQVYTLPPSRDELTKNQVSLTCLVKGFYPSDIAVEWESNGQPENNYKTTPPVLDSDGSFFLYSKLTVDKSRWQQGNVFSCSVMHEALHNHYTQKSLSCLSPGK

SEQ ID NO: 11 - DNA, 321 bp, LC-V205C Kappa DNA
acggtggctgcaccatctgtcttcatcttcccgccatctgatgagcagttgaaatctggaactgcctctgttgtgtgcctgctgaataacttctatcccagagaggccaaagtacagtggaaggtggataacgccctccaatcgggtaactcccaggagagtgtcacagagcaggacagcaaggacagcacctacagcctcagcagcaccctgacgctgagcaaagcagactacgagaaacacaaagtctacgcctgcgaagtcacccatcagggcctgagctcgccctgcacaaagagcttcaacaggggagagtgttag

SEQ ID NO: 12 - protein, 106 aa, LC-V205C Kappa
TVAAPSVFIFPPSDEQLKSGTASVVCLLNNFYPREAKVQWKVDNALQSGNSQESVTEQDSKDSTYSLSSTLTLSKADYEKHKVYACEVTHQGLSSPCTKSFNRGEC